European Patent Application EP 4 559 519 A1, published May 28, 2025. Title: Mutated human acidic chitinase for medical use. Applicant: Bioinova a.s. Application EP. The sequence listing filed with the application follows.

SEQUENCE LISTING (4 sequences)

SEQ ID NO: 1 - protein, 476 aa, Homo sapiens [sequence omitted]

SEQ ID NO: 2 - protein, 476 aa, synthetic construct
  VARIANT 45: note = N or D
  VARIANT 47: note = D or N
  VARIANT 102: note = G or R
  VARIANT 125: note = K or R
  VARIANT 339: note = V or I
  VARIANT 354: note = F or S
  VARIANT 432: note = G or V
MTKLILLTGLVLILNLQLGSAYQLTCYFTNWAQYRPGLGRFMPDNIDPCLCTHLIYAFAGMQNNEITTIEWNDVTLYQAFNGLKNKNSQLKTLLAIGGWNFGTAPFTAMVSTPENRQTFITSVIKFLRQYEFDGLDFDWEYPGSRGSPPQDKHLFTVLVQETREAFEQEAKQSNKPRLLVTAAVAAGISTIQSGYEIPQLSQYLDYIHVMTYDLHGSWEGYTGENSPLYKYPTDTGSNAYLNVDYAMNYWKNNGAPAEKLIVGFPTYGHTFLLSNPSNTGIGAPTSGAGPAGPYAKESGFWAYYEICTFLKNGATQGWDAPQEVPYAYQGNVWVGYDNIKSFDIKAQWLKHNKFGGAMVWAIDLDDFTGTFCNQGKFPLISTLKKALGLQSASCTAPAQPIEPITAAPSGSGNGSGSSSSGGSSGGSGFCAVRANGLYPVANNRNAFWHCVNGVTYQQNCQAGLVFDTSCDCCNWA

SEQ ID NO: 3 - protein, 455 aa, synthetic construct
  VARIANT 24: note = N or D
  VARIANT 26: note = D or N
  VARIANT 81: note = G or R
  VARIANT 104: note = K or R
  VARIANT 318: note = V or I
  VARIANT 333: note = F or S
  VARIANT 411: note = G or V
YQLTCYFTNWAQYRPGLGRFMPDNIDPCLCTHLIYAFAGMQNNEITTIEWNDVTLYQAFNGLKNKNSQLKTLLAIGGWNFGTAPFTAMVSTPENRQTFITSVIKFLRQYEFDGLDFDWEYPGSRGSPPQDKHLFTVLVQETREAFEQEAKQSNKPRLLVTAAVAAGISTIQSGYEIPQLSQYLDYIHVMTYDLHGSWEGYTGENSPLYKYPTDTGSNAYLNVDYAMNYWKNNGAPAEKLIVGFPTYGHTFLLSNPSNTGIGAPTSGAGPAGPYAKESGFWAYYEICTFLKNGATQGWDAPQEVPYAYQGNVWVGYDNIKSFDIKAQWLKHNKFGGAMVWAIDLDDFTGTFCNQGKFPLISTLKKALGLQSASCTAPAQPIEPITAAPSGSGNGSGSSSSGGSSGGSGFCAVRANGLYPVANNRNAFWHCVNGVTYQQNCQAGLVFDTSCDCCNWA

SEQ ID NO: 4 - protein, 21 aa, Homo sapiens
MTKLILLTGLVLILNLQLGSA